European Patent Application EP 4 445 949 A1, published October 16, 2024. Title: 脂肪肝炎用医薬. Applicant: 国立大学法人　東京大学. Application JP. The sequence listing filed with the application follows.

SEQUENCE LISTING (9 sequences)

SEQ ID NO: 1 - DNA, 20 bp, Mus musculus
  source 1..20: mol_type = genomic DNA
gcaagtgactcagacgtatg

SEQ ID NO: 2 - DNA, 20 bp, Mus musculus
  source 1..20: mol_type = genomic DNA
cagcttgtaagatcgccttg

SEQ ID NO: 3 - DNA, 43 bp, synthetic construct
  misc_feature 1..43: note = Synthetic primer
  source 1..43: mol_type = other DNA
cgggctgcaggaatttgatggctatttacattcccaccgtcta

SEQ ID NO: 4 - DNA, 28 bp, synthetic construct
  misc_feature 1..28: note = Synthetic primer
  source 1..28: mol_type = other DNA
acgcatgtttgaacgtcatgtctaattg

SEQ ID NO: 5 - DNA, 20 bp, synthetic construct
  misc_feature 1..20: note = Synthetic primer
  source 1..20: mol_type = other DNA
ttgccgggaagctagagtaa

SEQ ID NO: 6 - DNA, 20 bp, synthetic construct
  misc_feature 1..20: note = Synthetic primer
  source 1..20: mol_type = other DNA
tttgccttcctgtttttgct

SEQ ID NO: 7 - DNA, 20 bp, synthetic construct
  misc_feature 1..20: note = Synthetic DNA
  source 1..20: mol_type = other DNA
tagggaaccacttcgtcatt

SEQ ID NO: 8 - DNA, 24 bp, synthetic construct
  misc_feature 1..24: note = Synthetic primer
  source 1..24: mol_type = other DNA
gcagcatgcaggcagtattcaacc

SEQ ID NO: 9 - DNA, 24 bp, synthetic construct
  misc_feature 1..24: note = Synthetic primer
  source 1..24: mol_type = other DNA
cgagttcacaccactggactccag